European Patent Specification EP 3 560 502 B1, published September 24, 2025. Title: SMN2 Element 1 Antisense Compositions and Methods and Uses Thereof. Applicant: The Curators of the University of Missouri. The sequence listing filed with the application follows.

SEQUENCE LISTING (45 sequences)

SEQ ID NO: 1 - DNA, 222 bp, Homo sapiens
tgcaagaaaaccttaactgcagcctaataattgttttctttgggataacttttaaagtacattaaaagactatcaacttaatttctgatcatattttgttgaataaaataagtaaaatgtcttgtgaaacaaaatgctttttaacatccatataaagctatctatatatagctatctatgtctatatagctattttttttaacttcctttattttccttaca

SEQ ID NO: 2 - DNA, 45 bp, Homo sapiens
gtaaaatgtcttgtgaaacaaaatgctttttaacatccatataaa

SEQ ID NO: 3 - DNA, 87 bp, Homo sapiens
atattttgttgaataaaataagtaaaatgtcttgtgaaacaaaatgctttttaacatccatataaagctatctatatatagctatct

SEQ ID NO: 4 - DNA, 87 bp, Homo sapiens
tctatcgatatatatctatcgaaatatacctacaatttttcgtaaaacaaagtgttctgtaaaatgaataaaataagttgttttata

SEQ ID NO: 5 - DNA, 39 bp, Homo sapiens
ctatatatagatagttattcaacaaaactagtaattttt

SEQ ID NO: 6 - DNA, 26 bp, Homo sapiens
ctatatatagatagttattcaacaaa

SEQ ID NO: 7 - DNA, 25 bp, Homo sapiens
tagatagctttacattttacttatt

SEQ ID NO: 8 - DNA, 25 bp, Homo sapiens
tatggatgttaaaaagcattttgtt

SEQ ID NO: 9 - DNA, 25 bp, Homo sapiens
ctatatatagatagctttatatgga

SEQ ID NO: 10 - DNA, 25 bp, Homo sapiens
cattttacttattttattcaacaaa

SEQ ID NO: 11 - DNA, 25 bp, Homo sapiens
gctttatatggacattttacttatt

SEQ ID NO: 12 - DNA, 25 bp, Homo sapiens
gatgttaaaaagcgtttcacaagac

SEQ ID NO: 13 - DNA, 25 bp, Homo sapiens
tatatggatgttattattcaacaaa

SEQ ID NO: 14 - DNA, 25 bp, Homo sapiens
gcattttgtttcacaagttattcaa

SEQ ID NO: 15 - DNA, 25 bp, Homo sapiens
ctatatatagatagcgacattttac

SEQ ID NO: 16 - DNA, 26 bp, Homo sapiens
agatagctttatatggatttattcaa

SEQ ID NO: 17 - DNA, 20 bp, Homo sapiens
ctatatatagttattcaaca

SEQ ID NO: 18 - DNA, 24 bp, Homo sapiens
tttatatggatgaagacattttac

SEQ ID NO: 19 - DNA, 24 bp, Mus musculus
tctgtgttcgtgcgtggtgacttt

SEQ ID NO: 20 - DNA, 24 bp, Mus musculus
cccaccacctaagaaagcctcaat

SEQ ID NO: 21 - DNA, 24 bp, Mus musculus
ccaacttaatcgccttgcagcaca

SEQ ID NO: 22 - DNA, 24 bp, Mus musculus
aagcgagtggcaacatggaaatcg

SEQ ID NO: 23 - RNA, 25 nt, Artificial Sequence
  Synthetic
ccucuuaccucaguuacaauuuaua

SEQ ID NO: 24 - RNA, 26 nt, Homo sapiens
cuauauauagauaguuauucaacaaa

SEQ ID NO: 25 - RNA, 14 nt, Homo sapiens
cuauauauagauag

SEQ ID NO: 26 - RNA, 12 nt, Homo sapiens
uuauucaacaaa

SEQ ID NO: 27 - RNA, 15 nt, Homo sapiens
cuuucauaaugcugg

SEQ ID NO: 28 - RNA, 18 nt, Homo sapiens
ucacuuucauaaugcugg

SEQ ID NO: 29 - RNA, 20 nt, Homo sapiens
auucacuuucauaaugcugg

SEQ ID NO: 30 - RNA, 20 nt, Homo sapiens
auucacuuucauaaugcugg

SEQ ID NO: 31 - RNA, 21 nt, Homo sapiens
gauucacuuucauaaugcugg

SEQ ID NO: 32 - RNA, 25 nt, Homo sapiens
guuagauucacuuucauaaugcugg

SEQ ID NO: 33 - DNA, 87 bp, Homo sapiens; identical to SEQ ID NO: 3

SEQ ID NO: 34 - DNA, 87 bp, Homo sapiens; identical to SEQ ID NO: 3

SEQ ID NO: 35 - DNA, 87 bp, Homo sapiens; identical to SEQ ID NO: 3

SEQ ID NO: 36 - DNA, 87 bp, Homo sapiens; identical to SEQ ID NO: 3

SEQ ID NO: 37 - DNA, 87 bp, Homo sapiens; identical to SEQ ID NO: 3

SEQ ID NO: 38 - DNA, 87 bp, Homo sapiens; identical to SEQ ID NO: 3

SEQ ID NO: 39 - DNA, 87 bp, Homo sapiens; identical to SEQ ID NO: 3

SEQ ID NO: 40 - DNA, 87 bp, Homo sapiens; identical to SEQ ID NO: 3

SEQ ID NO: 41 - DNA, 87 bp, Homo sapiens; identical to SEQ ID NO: 3

SEQ ID NO: 42 - DNA, 87 bp, Homo sapiens; identical to SEQ ID NO: 3

SEQ ID NO: 43 - DNA, 87 bp, Homo sapiens; identical to SEQ ID NO: 3

SEQ ID NO: 44 - DNA, 87 bp, Homo sapiens; identical to SEQ ID NO: 3

SEQ ID NO: 45 - DNA, 87 bp, Homo sapiens; identical to SEQ ID NO: 3